European Patent Application EP 4 227 321 A1, published August 16, 2023. Title: ANTIBODIES TARGETING THE B-CELL RECEPTOR OF CHRONIC LYMPHOCYTIC LEUKEMIA AND USES THEREOF. Applicant: AVA Lifescience GmbH. The sequence listing filed with the application follows.

SEQUENCE LISTING (53 sequences)

SEQ ID NO: 1 - protein, 443 aa, Mus musculus
QVQLQQSGPGLVQPSQSLSITCTVSGFSLTSYGIHWVRQSPGKGLEWLGVIWRGGGTDSNAAFMSRLSITKDNSKSQVFFKMNSLQADDTAIYYCARSRYDEEESMNYWGQGTSVTVSSAKTTPPSVYPLAPGSAAQTNSMVTLGCLVKGYFPEPVTVTWNSGSLSSGVHTFPAVLQSDLYTLSSSVTVPSSPRPSETVTCNVAHPASSTKVDKKIVPRDCGCKPCICTVPEVSSVFIFPPKPKDVLTITLTPKVTCVVVDISKDDPEVQFSWFVDDVEVHTAQTQPREEQFNSTFRSVSELPIMHQDWLNGKEFKCRVNSAAFPAPIEKTISKTKGRPKAPQVYTIPPPKEQMAKDKVSLTCMITDFFPEDITVEWQWNGQPAENYKNTQPIMNTNGSYFVYSKLNVQKSNWEAGNTFTCSVLHEGLHNHHTEKSLSHSPGK

SEQ ID NO: 2 - protein, 214 aa, Mus musculus
QIVLTQSPASLSASVGETVTITCRASGNIHSYLAWYQQKQGKSPQLLVYNAKTLADGVPSRFSGSGSGTQYSLKINSLQPEDFGSYYCQHFWNTPPTFGAGTKLELKRADAAPTVSIFPPSSEQLTSGGASVVCFLNNFYPKDINVKWKIDGSERQNGVLNSWTDQDSKDSTYSMSSTLTLTKDEYERHNSYTCEATHKTSTSPIVKSFNRNEC

SEQ ID NO: 3 - protein, 119 aa, Mus musculus
QVQLQQSGPGLVQPSQSLSITCTVSGFSLTSYGIHWVRQSPGKGLEWLGVIWRGGGTDSNAAFMSRLSITKDNSKSQVFFKMNSLQADDTAIYYCARSRYDEEESMNYWGQGTSVTVSS

SEQ ID NO: 4 - protein, 108 aa, Mus musculus
QIVLTQSPASLSASVGETVTITCRASGNIHSYLAWYQQKQGKSPQLLVYNAKTLADGVPSRFSGSGSGTQYSLKINSLQPEDFGSYYCQHFWNTPPTFGAGTKLELKR

SEQ ID NO: 5 - protein, 8 aa, Mus musculus
GFSLTSYG

SEQ ID NO: 6 - protein, 7 aa, Mus musculus
IWRGGGT

SEQ ID NO: 7 - protein, 13 aa, Mus musculus
ARSRYDEEESMNY

SEQ ID NO: 8 - protein, 6 aa, Mus musculus
GNIHSY

SEQ ID NO: 9 - protein, 4 aa, Mus musculus
NAKT

SEQ ID NO: 10 - protein, 9 aa, Mus musculus
QHFWNTPPT

SEQ ID NO: 11 - protein, 449 aa, Artificial Sequence
  Synthetic polypeptide
QVQLQQSGPGLVQPSQSLSITCTVSGFSLTSYGIHWVRQSPGKGLEWLGVIWRGGGTDSNAAFMSRLSITKDNSKSQVFFKMNSLQADDTAIYYCARSRYDEEESMNYWGQGTSVTVSSASTKGPSVFPLAPSSKSTSGGTAALGCLVKDYFPEPVTVSWNSGALTSGVHTFPAVLQSSGLYSLSSVVTVPSSSLGTQTYICNVNHKPSNTKVDKKVEPKSCDKTHTCPPCPAPELLGGPSVFLFPPKPKDTLMISRTPEVTCVVVDVSHEDPEVKFNWYVDGVEVHNAKTKPREEQYNSTYRVVSVLTVLHQDWLNGKEYKCKVSNKALPAPIEKTISKAKGQPREPQVYTLPPSRDELTKNQVSLTCLVKGFYPSDIAVEWESNGQPENNYKTTPPVLDSDGSFFLYSKLTVDKSRWQQGNVFSCSVMHEALHNHYTQKSLSLSPGK

SEQ ID NO: 12 - protein, 214 aa, Artificial Sequence
  Synthetic polypeptide
QIVLTQSPASLSASVGETVTITCRASGNIHSYLAWYQQKQGKSPQLLVYNAKTLADGVPSRFSGSGSGTQYSLKINSLQPEDFGSYYCQHFWNTPPTFGAGTKLELKRTVAAPSVFIFPPSDEQLKSGTASVVCLLNNFYPREAKVQWKVDNALQSGNSQESVTEQDSKDSTYSLSSTLTLSKADYEKHKVYACEVTHQGLSSPVTKSFNRGEC

SEQ ID NO: 13 - protein, 449 aa, Artificial Sequence
  Synthetic polypeptide
QVQLQESGPGLVKPSETLSLTCTVSGFSLTSYGIHWIRQSPGRGLEWIGVIWRGGGTDSNAAFMSRITISRDTSKTQVSLKLGSVTAADTAIYYCARSRYDEEESMNYWGQGTSVTVSSASTKGPSVFPLAPSSKSTSGGTAALGCLVKDYFPEPVTVSWNSGALTSGVHTFPAVLQSSGLYSLSSVVTVPSSSLGTQTYICNVNHKPSNTKVDKKVEPKSCDKTHTCPPCPAPELLGGPSVFLFPPKPKDTLMISRTPEVTCVVVDVSHEDPEVKFNWYVDGVEVHNAKTKPREEQYNSTYRVVSVLTVLHQDWLNGKEYKCKVSNKALPAPIEKTISKAKGQPREPQVYTLPPSRDELTKNQVSLTCLVKGFYPSDIAVEWESNGQPENNYKTTPPVLDSDGSFFLYSKLTVDKSRWQQGNVFSCSVMHEALHNHYTQKSLSLSPGK

SEQ ID NO: 14 - protein, 214 aa, Artificial Sequence
  Synthetic polypeptide
EIVLTQSPSSLSASVGDSVTITCRASGNIHSYLAWYQQKPGKAPKLLIYNAKTLADGVPSRFSGSGSGTQYTLTISSLQPEDFATYYCQHFWNTPPTFGAGTKLELKRTVAAPSVFIFPPSDEQLKSGTASVVCLLNNFYPREAKVQWKVDNALQSGNSQESVTEQDSKDSTYSLSSTLTLSKADYEKHKVYACEVTHQGLSSPVTKSFNRGEC

SEQ ID NO: 15 - protein, 119 aa, Artificial Sequence
  Synthetic polypeptide
QVQLQESGPGLVKPSETLSLTCTVSGFSLTSYGIHWIRQSPGRGLEWIGVIWRGGGTDSNAAFMSRITISRDTSKTQVSLKLGSVTAADTAIYYCARSRYDEEESMNYWGQGTSVTVSS

SEQ ID NO: 16 - protein, 108 aa, Artificial Sequence
  Synthetic polypeptide
EIVLTQSPSSLSASVGDSVTITCRASGNIHSYLAWYQQKPGKAPKLLIYNAKTLADGVPSRFSGSGSGTQYTLTISSLQPEDFATYYCQHFWNTPPTFGAGTKLELKR

SEQ ID NO: 17 - protein, 108 aa, Artificial Sequence
  Synthetic polypeptide
QIQLTQSPSFLSASVGDSVTITCRASGNIHSYLAWYQQKPGKAPQLLIYNAKTLADGVPSRFSGSGSGTEYTLTISSLQPEDFATYYCQHFWNTPPTFGAGTKLELKR

SEQ ID NO: 18 - protein, 108 aa, Artificial Sequence
  Synthetic polypeptide
EIVLTQSPATLSLSPGERATLSCRASGNIHSYLAWYQQKPGQAPRLLIYNAKTLADGIPARFSGSGSGTDYTLTISSLEPEDFASYYCQHFWNTPPTFGAGTKLELKR

SEQ ID NO: 19 - protein, 108 aa, Artificial Sequence
  Synthetic polypeptide
EIVLTQSPGTLSLSPGERATLSCRASGNIHSYLAWYQQKPGQAPRLLIYNAKTLADGIPDRFSGSGSGTDYTLTISRLEPEDFAVYYCQHFWNTPPTFGAGTKLELKR

SEQ ID NO: 20 - protein, 119 aa, Artificial Sequence; identical to SEQ ID NO: 15
  Synthetic polypeptide

SEQ ID NO: 21 - protein, 449 aa, Artificial Sequence; identical to SEQ ID NO: 13
  Synthetic polypeptide

SEQ ID NO: 22 - protein, 214 aa, Artificial Sequence
  Synthetic polypeptide
QIQLTQSPSFLSASVGDSVTITCRASGNIHSYLAWYQQKPGKAPQLLIYNAKTLADGVPSRFSGSGSGTEYTLTISSLQPEDFATYYCQHFWNTPPTFGAGTKLELKRTVAAPSVFIFPPSDEQLKSGTASVVCLLNNFYPREAKVQWKVDNALQSGNSQESVTEQDSKDSTYSLSSTLTLSKADYEKHKVYACEVTHQGLSSPVTKSFNRGEC

SEQ ID NO: 23 - protein, 214 aa, Artificial Sequence
  Synthetic polypeptide
EIVLTQSPATLSLSPGERATLSCRASGNIHSYLAWYQQKPGQAPRLLIYNAKTLADGIPARFSGSGSGTDYTLTISSLEPEDFASYYCQHFWNTPPTFGAGTKLELKRTVAAPSVFIFPPSDEQLKSGTASVVCLLNNFYPREAKVQWKVDNALQSGNSQESVTEQDSKDSTYSLSSTLTLSKADYEKHKVYACEVTHQGLSSPVTKSFNRGEC

SEQ ID NO: 24 - protein, 214 aa, Artificial Sequence
  Synthetic polypeptide
EIVLTQSPGTLSLSPGERATLSCRASGNIHSYLAWYQQKPGQAPRLLIYNAKTLADGIPDRFSGSGSGTDYTLTISRLEPEDFAVYYCQHFWNTPPTFGAGTKLELKRTVAAPSVFIFPPSDEQLKSGTASVVCLLNNFYPREAKVQWKVDNALQSGNSQESVTEQDSKDSTYSLSSTLTLSKADYEKHKVYACEVTHQGLSSPVTKSFNRGEC

SEQ ID NO: 25 - DNA, 1329 bp, Mus musculus
caggtgcagctgcagcagtctggacctggcctagtgcagccctcacagagcctgtccataacctgcacagtctctggtttctcattaactagctatggtatacactgggttcgccagtctccaggaaagggtctggagtggctgggagtgatatggagaggtggaggcacagactccaatgcagctttcatgtccagactgagcatcaccaaggacaattccaagagccaagttttctttaaaatgaacagtctgcaagctgatgacactgccatatattactgtgccagaagtaggtacgacgaggaggaaagtatgaactactggggtcaaggaacctcagtcaccgtctcctcagccaaaacgacacccccatctgtctatccactggcccctggatctgctgcccaaactaactccatggtgaccctgggatgcctggtcaagggctatttccctgagccagtgacagtgacctggaactctggatccctgtccagcggtgtgcacaccttcccagctgtcctgcagtctgacctctacactctgagcagctcagtgactgtcccctccagccctcggcccagcgagaccgtcacctgcaacgttgcccacccggccagcagcaccaaggtggacaagaaaattgtgcccagggattgtggttgtaagccttgcatatgtacagtcccagaagtatcatctgtcttcatcttccccccaaagcccaaggatgtgctcaccattactctgactcctaaggtcacgtgtgttgtggtagacatcagcaaggatgatcccgaggtccagttcagctggtttgtagatgatgtggaggtgcacacagctcagacgcaaccccgggaggagcagttcaacagcactttccgctcagtcagtgaacttcccatcatgcaccaggactggctcaatggcaaggagttcaaatgcagggtcaacagtgcagctttccctgcccccatcgagaaaaccatctccaaaaccaaaggcagaccgaaggctccacaggtgtacaccattccacctcccaaggagcagatggccaaggataaagtcagtctgacctgcatgataacagacttcttccctgaagacattactgtggagtggcagtggaatgggcagccagcggagaactacaagaacactcagcccatcatgaacacgaatggctcttacttcgtctacagcaagctcaatgtgcagaagagcaactgggaggcaggaaatactttcacctgctctgtgttacatgagggcctgcacaaccaccatactgagaagagcctctcccactctcctggtaaa

SEQ ID NO: 26 - DNA, 642 bp, Mus musculus
caaattgttctcacccagtctccagcctccctatctgcatctgtgggagaaactgtcaccatcacttgtcgagcaagtgggaatattcacagttatttagcatggtatcagcagaaacagggaaaatctcctcagctcctggtctataatgcaaaaaccttagcagatggtgtgccatcaaggttcagtggcagtggatcaggaacacaatattctctcaagatcaacagcctgcagcctgaagattttgggagttattactgtcaacatttttggaatactcctcccacgttcggtgctgggaccaagctggagctgaaacgggctgatgctgcaccaactgtatccatcttcccaccatccagtgagcagttaacatctggaggtgcctcagtcgtgtgcttcttgaacaacttctaccccaaagacatcaatgtcaagtggaagattgatggcagtgaacgacaaaatggcgtcctgaacagttggactgatcaggacagcaaagacagcacctacagcatgagcagcaccctcacgttgaccaaggacgagtatgaacgacataacagctatacctgtgaggccactcacaagacatcaacttcacccattgtcaagagcttcaacaggaatgagtgt

SEQ ID NO: 27 - DNA, 357 bp, Mus musculus
caggtgcagctgcagcagtctggacctggcctagtgcagccctcacagagcctgtccataacctgcacagtctctggtttctcattaactagctatggtatacactgggttcgccagtctccaggaaagggtctggagtggctgggagtgatatggagaggtggaggcacagactccaatgcagctttcatgtccagactgagcatcaccaaggacaattccaagagccaagttttctttaaaatgaacagtctgcaagctgatgacactgccatatattactgtgccagaagtaggtacgacgaggaggaaagtatgaactactggggtcaaggaacctcagtcaccgtctcctca

SEQ ID NO: 28 - protein, 321 aa, Mus musculus
CAAATTGTTCTCACCCAGTCTCCAGCCTCCCTATCTGCATCTGTGGGAGAAACTGTCACCATCACTTGTCGAGCAAGTGGGAATATTCACAGTTATTTAGCATGGTATCAGCAGAAACAGGGAAAATCTCCTCAGCTCCTGGTCTATAATGCAAAAACCTTAGCAGATGGTGTGCCATCAAGGTTCAGTGGCAGTGGATCAGGAACACAATATTCTCTCAAGATCAACAGCCTGCAGCCTGAAGATTTTGGGAGTTATTACTGTCAACATTTTTGGAATACTCCTCCCACGTTCGGTGCTGGGACCAAGCTGGAGCTGAAA

SEQ ID NO: 29 - DNA, 1347 bp, Artificial Sequence
  Synthetic polynucleotide
caggtgcagctgcagcagtctggacctggcctagtgcagccctcacagagcctgtccataacctgcacagtctctggtttctcattaactagctatggtatacactgggttcgccagtctccaggaaagggtctggagtggctgggagtgatatggagaggtggaggcacagactccaatgcagctttcatgtccagactgagcatcaccaaggacaattccaagagccaagttttctttaaaatgaacagtctgcaagctgatgacactgccatatattactgtgccagaagtaggtacgacgaggaggaaagtatgaactactggggtcaaggaacctcagtcaccgtctcctcagccagcaccaagggccccagcgtgttccccctggcccccagcagcaagagcaccagcggcggcaccgccgccctgggctgcctggtgaaggactacttccccgagcccgtgaccgtgagctggaacagcggcgccctgaccagcggcgtgcacaccttccccgccgtgctgcagagcagcggcctgtacagcctgagcagcgtggtgaccgtgcccagcagcagcctgggcacccagacctacatctgcaacgtgaaccacaagcccagcaacaccaaggtggacaagaaggtggagcccaagagctgcgacaagacccacacctgccccccctgccccgcccccgagctgctgggcggccccagcgtgttcctgttcccccccaagcccaaggacaccctgatgatcagcaggacccccgaggtgacctgcgtggtggtggacgtgagccacgaggaccccgaggtgaagttcaactggtacgtggacggcgtggaggtgcacaacgccaagaccaagcccagggaggagcagtacaacagcacctacagggtggtgagcgtgctgaccgtgctgcaccaggactggctgaacggcaaggagtacaagtgcaaggtgagcaacaaggccctgcccgcccccatcgagaagaccatcagcaaggccaagggccagcccagggagccccaggtgtacaccctgccccccagcagggacgagctgaccaagaaccaggtgagcctgacctgcctggtgaagggcttctaccccagcgacatcgccgtggagtgggagagcaacggccagcccgagaacaactacaagaccaccccccccgtgctggacagcgacggcagcttcttcctgtacagcaagctgaccgtggacaagagcaggtggcagcagggcaacgtgttcagctgcagcgtgatgcacgaggccctgcacaaccactacacccagaagagcctgagcctgagccccggcaag

SEQ ID NO: 30 - DNA, 642 bp, Artificial Sequence
  Synthetic polynucleotide
caaattgttctcacccagtctccagcctccctatctgcatctgtgggagaaactgtcaccatcacttgtcgagcaagtgggaatattcacagttatttagcatggtatcagcagaaacagggaaaatctcctcagctcctggtctataatgcaaaaaccttagcagatggtgtgccatcaaggttcagtggcagtggatcaggaacacaatattctctcaagatcaacagcctgcagcctgaagattttgggagttattactgtcaacatttttggaatactcctcccacgttcggtgctgggaccaagctggagctgaaacgcaccgtggcggcgccgagcgtgtttatttttccgccgagcgatgaacagctgaaaagcggcaccgcgagcgtggtgtgcctgctgaacaacttttatccgcgcgaagcgaaagtgcagtggaaagtggataacgcgctgcagagcggcaacagccaggaaagcgtgaccgaacaggatagcaaagatagcacctatagcctgagcagcaccctgaccctgagcaaagcggattatgaaaaacataaagtgtatgcgtgcgaagtgacccatcagggcctgagcagcccggtgaccaaaagctttaaccgcggcgaatgc

SEQ ID NO: 31 - DNA, 990 bp, Homo sapiens
gccagcaccaagggccccagcgtgttccccctggcccccagcagcaagagcaccagcggcggcaccgccgccctgggctgcctggtgaaggactacttccccgagcccgtgaccgtgagctggaacagcggcgccctgaccagcggcgtgcacaccttccccgccgtgctgcagagcagcggcctgtacagcctgagcagcgtggtgaccgtgcccagcagcagcctgggcacccagacctacatctgcaacgtgaaccacaagcccagcaacaccaaggtggacaagaaggtggagcccaagagctgcgacaagacccacacctgccccccctgccccgcccccgagctgctgggcggccccagcgtgttcctgttcccccccaagcccaaggacaccctgatgatcagcaggacccccgaggtgacctgcgtggtggtggacgtgagccacgaggaccccgaggtgaagttcaactggtacgtggacggcgtggaggtgcacaacgccaagaccaagcccagggaggagcagtacaacagcacctacagggtggtgagcgtgctgaccgtgctgcaccaggactggctgaacggcaaggagtacaagtgcaaggtgagcaacaaggccctgcccgcccccatcgagaagaccatcagcaaggccaagggccagcccagggagccccaggtgtacaccctgccccccagcagggacgagctgaccaagaaccaggtgagcctgacctgcctggtgaagggcttctaccccagcgacatcgccgtggagtgggagagcaacggccagcccgagaacaactacaagaccaccccccccgtgctggacagcgacggcagcttcttcctgtacagcaagctgaccgtggacaagagcaggtggcagcagggcaacgtgttcagctgcagcgtgatgcacgaggccctgcacaaccactacacccagaagagcctgagcctgagccccggcaag

SEQ ID NO: 32 - DNA, 321 bp, Homo sapiens
cgcaccgtggcggcgccgagcgtgtttatttttccgccgagcgatgaacagctgaaaagcggcaccgcgagcgtggtgtgcctgctgaacaacttttatccgcgcgaagcgaaagtgcagtggaaagtggataacgcgctgcagagcggcaacagccaggaaagcgtgaccgaacaggatagcaaagatagcacctatagcctgagcagcaccctgaccctgagcaaagcggattatgaaaaacataaagtgtatgcgtgcgaagtgacccatcagggcctgagcagcccggtgaccaaaagctttaaccgcggcgaatgc

SEQ ID NO: 33 - DNA, 357 bp, Artificial Sequence
  Synthetic polynucleotide
caggtgcagctgcaggagagcggccccggcctggtgaagcccagcgagaccctgagcctgacctgcaccgtgagcggcttcagcctgaccagctacggcatccactggatcaggcagagccccggcaggggcctggagtggatcggcgtgatctggaggggcggcggcaccgacagcaacgccgccttcatgagcagggtgaccatcagcagggacaccagcaagagccaggtgagcctgaagctgggcagcgtgaccgccgccgacaccgccatctactactgcgccaggagcaggtacgacgaggaggagagcatgaactactggggccagggcaccagcgtgaccgtgagcagc

SEQ ID NO: 34 - DNA, 321 bp, Artificial Sequence
  Synthetic polynucleotide
gaaattgtgctgacccagagcccgagcagcctgagcgcgagcgtgggcgatagcgtgaccattacctgccgcgcgagcggcaacattcatagctatctggcgtggtatcagcagaaaccgggcaaagcgccgaaactgctgatttataacgcgaaaaccctggcggatggcgtgccgagccgctttagcggcagcggcagcggcacccagtataccctgaccattagcagcctgcagccggaagattttgcgacctattattgccagcatttttggaacaccccgccgacctttggcgcgggcaccaaactggaactgaaa

SEQ ID NO: 35 - DNA, 321 bp, Artificial Sequence
  Synthetic polynucleotide
cagattcagctgacccagagcccgagctttctgagcgcgagcgtgggcgatagcgtgaccattacctgccgcgcgagcggcaacattcatagctatctggcgtggtatcagcagaaaccgggcaaagcgccgcagctgctgatttataacgcgaaaaccctggcggatggcgtgccgagccgctttagcggcagcggcagcggcaccgaatataccctgaccattagcagcctgcagccggaagattttgcgacctattattgccagcatttttggaacaccccgccgacctttggcgcgggcaccaaactggaactgaaa

SEQ ID NO: 36 - DNA, 321 bp, Artificial Sequence
  Synthetic polynucleotide
gagatcgtgctgacccagagccccgccaccctgagcctgagccccggcgagagggccaccctgagctgcagggccagcggcaacatccacagctacctggcctggtaccagcagaagcccggccaggcccccaggctgctgatctacaacgccaagaccctggccgacggcatccccgccaggttcagcggcagcggcagcggcaccgactacaccctgaccatcagcagcctggagcccgaggacttcgccagctactactgccagcacttctggaacaccccccccaccttcggcgccggcaccaagctggagctgaag

SEQ ID NO: 37 - DNA, 321 bp, Artificial Sequence
  Synthetic polynucleotide
gagatcgtgctgacccagagccccggcaccctgagcctgagccccggcgagagggccaccctgagctgcagggccagcggcaacatccacagctacctggcctggtaccagcagaagcccggccaggcccccaggctgctgatctacaacgccaagaccctggccgacggcatccccgacaggttcagcggcagcggcagcggcaccgactacaccctgaccatcagcaggctggagcccgaggacttcgccgtgtactactgccagcacttctggaacaccccccccaccttcggcgccggcaccaagctggagctgaag

SEQ ID NO: 38 - DNA, 357 bp, Artificial Sequence
  Synthetic polynucleotide
caggtgcagctgcaggagagcggccccggcctggtgaagcccagcgagaccctgagcctgacctgcaccgtgagcggcttcagcctgaccagctacggcatccactggatcaggcagagccccggcaggggcctggagtggatcggcgtgatctggaggggcggcggcaccgacagcaacgccgccttcatgagcaggatcaccatcagcagggacaccagcaagacccaggtgagcctgaagctgggcagcgtgaccgccgccgacaccgccatctactactgcgccaggagcaggtacgacgaggaggagagcatgaactactggggccagggcaccagcgtgaccgtgagcagc

SEQ ID NO: 39 - protein, 657 aa, Artificial Sequence
  Synthetic polypeptide
QVQLQQSGPGLVQPSQSLSITCTVSGFSLTSYGIHWVRQSPGKGLEWLGVIWRGGGTDSNAAFMSRLSITKDNSKSQVFFKMNSLQADDTAIYYCARSRYDEEESMNYWGQGTSVTVSSAKTTPPSVYPLAPGSAAQTNSMVTLGCLVKGYFPEPVTVTWNSGSLSSGVHTFPAVLQSDLYTLSSSVTVPSSPRPSETVTCNVAHPASSTKVDKKIVPRDCGCKPCICTVPEVSSVFIFPPKPKDVLTITLTPKVTCVVVDISKDDPEVQFSWFVDDVEVHTAQTQPREEQFNSTFRSVSELPIMHQDWLNGKEFKCRVNSAAFPAPIEKTISKTKGRPKAPQVYTIPPPKEQMAKDKVSLTCMITDFFPEDITVEWQWNGQPAENYKNTQPIMNTNGSYFVYSKLNVQKSNWEAGNTFTCSVLHEGLHNHHTEKSLSHSPGKQIVLTQSPASLSASVGETVTITCRASGNIHSYLAWYQQKQGKSPQLLVYNAKTLADGVPSRFSGSGSGTQYSLKINSLQPEDFGSYYCQHFWNTPPTFGAGTKLELKRADAAPTVSIFPPSSEQLTSGGASVVCFLNNFYPKDINVKWKIDGSERQNGVLNSWTDQDSKDSTYSMSSTLTLTKDEYERHNSYTCEATHKTSTSPIVKSFNRNEC

SEQ ID NO: 40 - protein, 663 aa, Artificial Sequence
  Synthetic polypeptide
QVQLQQSGPGLVQPSQSLSITCTVSGFSLTSYGIHWVRQSPGKGLEWLGVIWRGGGTDSNAAFMSRLSITKDNSKSQVFFKMNSLQADDTAIYYCARSRYDEEESMNYWGQGTSVTVSSASTKGPSVFPLAPSSKSTSGGTAALGCLVKDYFPEPVTVSWNSGALTSGVHTFPAVLQSSGLYSLSSVVTVPSSSLGTQTYICNVNHKPSNTKVDKKVEPKSCDKTHTCPPCPAPELLGGPSVFLFPPKPKDTLMISRTPEVTCVVVDVSHEDPEVKFNWYVDGVEVHNAKTKPREEQYNSTYRVVSVLTVLHQDWLNGKEYKCKVSNKALPAPIEKTISKAKGQPREPQVYTLPPSRDELTKNQVSLTCLVKGFYPSDIAVEWESNGQPENNYKTTPPVLDSDGSFFLYSKLTVDKSRWQQGNVFSCSVMHEALHNHYTQKSLSLSPGKQIVLTQSPASLSASVGETVTITCRASGNIHSYLAWYQQKQGKSPQLLVYNAKTLADGVPSRFSGSGSGTQYSLKINSLQPEDFGSYYCQHFWNTPPTFGAGTKLELKRTVAAPSVFIFPPSDEQLKSGTASVVCLLNNFYPREAKVQWKVDNALQSGNSQESVTEQDSKDSTYSLSSTLTLSKADYEKHKVYACEVTHQGLSSPVTKSFNRGEC

SEQ ID NO: 41 - protein, 663 aa, Artificial Sequence
  Synthetic polypeptide
QVQLQESGPGLVKPSETLSLTCTVSGFSLTSYGIHWIRQSPGRGLEWIGVIWRGGGTDSNAAFMSRITISRDTSKTQVSLKLGSVTAADTAIYYCARSRYDEEESMNYWGQGTSVTVSSASTKGPSVFPLAPSSKSTSGGTAALGCLVKDYFPEPVTVSWNSGALTSGVHTFPAVLQSSGLYSLSSVVTVPSSSLGTQTYICNVNHKPSNTKVDKKVEPKSCDKTHTCPPCPAPELLGGPSVFLFPPKPKDTLMISRTPEVTCVVVDVSHEDPEVKFNWYVDGVEVHNAKTKPREEQYNSTYRVVSVLTVLHQDWLNGKEYKCKVSNKALPAPIEKTISKAKGQPREPQVYTLPPSRDELTKNQVSLTCLVKGFYPSDIAVEWESNGQPENNYKTTPPVLDSDGSFFLYSKLTVDKSRWQQGNVFSCSVMHEALHNHYTQKSLSLSPGKEIVLTQSPSSLSASVGDSVTITCRASGNIHSYLAWYQQKPGKAPKLLIYNAKTLADGVPSRFSGSGSGTQYTLTISSLQPEDFATYYCQHFWNTPPTFGAGTKLELKRTVAAPSVFIFPPSDEQLKSGTASVVCLLNNFYPREAKVQWKVDNALQSGNSQESVTEQDSKDSTYSLSSTLTLSKADYEKHKVYACEVTHQGLSSPVTKSFNRGEC

SEQ ID NO: 42 - protein, 663 aa, Artificial Sequence
  Synthetic polypeptide
QVQLQESGPGLVKPSETLSLTCTVSGFSLTSYGIHWIRQSPGRGLEWIGVIWRGGGTDSNAAFMSRITISRDTSKTQVSLKLGSVTAADTAIYYCARSRYDEEESMNYWGQGTSVTVSSASTKGPSVFPLAPSSKSTSGGTAALGCLVKDYFPEPVTVSWNSGALTSGVHTFPAVLQSSGLYSLSSVVTVPSSSLGTQTYICNVNHKPSNTKVDKKVEPKSCDKTHTCPPCPAPELLGGPSVFLFPPKPKDTLMISRTPEVTCVVVDVSHEDPEVKFNWYVDGVEVHNAKTKPREEQYNSTYRVVSVLTVLHQDWLNGKEYKCKVSNKALPAPIEKTISKAKGQPREPQVYTLPPSRDELTKNQVSLTCLVKGFYPSDIAVEWESNGQPENNYKTTPPVLDSDGSFFLYSKLTVDKSRWQQGNVFSCSVMHEALHNHYTQKSLSLSPGKQIQLTQSPSFLSASVGDSVTITCRASGNIHSYLAWYQQKPGKAPQLLIYNAKTLADGVPSRFSGSGSGTEYTLTISSLQPEDFATYYCQHFWNTPPTFGAGTKLELKRTVAAPSVFIFPPSDEQLKSGTASVVCLLNNFYPREAKVQWKVDNALQSGNSQESVTEQDSKDSTYSLSSTLTLSKADYEKHKVYACEVTHQGLSSPVTKSFNRGEC

SEQ ID NO: 43 - protein, 663 aa, Artificial Sequence
  Synthetic polypeptide
QVQLQESGPGLVKPSETLSLTCTVSGFSLTSYGIHWIRQSPGRGLEWIGVIWRGGGTDSNAAFMSRITISRDTSKTQVSLKLGSVTAADTAIYYCARSRYDEEESMNYWGQGTSVTVSSASTKGPSVFPLAPSSKSTSGGTAALGCLVKDYFPEPVTVSWNSGALTSGVHTFPAVLQSSGLYSLSSVVTVPSSSLGTQTYICNVNHKPSNTKVDKKVEPKSCDKTHTCPPCPAPELLGGPSVFLFPPKPKDTLMISRTPEVTCVVVDVSHEDPEVKFNWYVDGVEVHNAKTKPREEQYNSTYRVVSVLTVLHQDWLNGKEYKCKVSNKALPAPIEKTISKAKGQPREPQVYTLPPSRDELTKNQVSLTCLVKGFYPSDIAVEWESNGQPENNYKTTPPVLDSDGSFFLYSKLTVDKSRWQQGNVFSCSVMHEALHNHYTQKSLSLSPGKEIVLTQSPATLSLSPGERATLSCRASGNIHSYLAWYQQKPGQAPRLLIYNAKTLADGIPARFSGSGSGTDYTLTISSLEPEDFASYYCQHFWNTPPTFGAGTKLELKRTVAAPSVFIFPPSDEQLKSGTASVVCLLNNFYPREAKVQWKVDNALQSGNSQESVTEQDSKDSTYSLSSTLTLSKADYEKHKVYACEVTHQGLSSPVTKSFNRGEC

SEQ ID NO: 44 - protein, 663 aa, Artificial Sequence
  Synthetic polypeptide
QVQLQESGPGLVKPSETLSLTCTVSGFSLTSYGIHWIRQSPGRGLEWIGVIWRGGGTDSNAAFMSRITISRDTSKTQVSLKLGSVTAADTAIYYCARSRYDEEESMNYWGQGTSVTVSSASTKGPSVFPLAPSSKSTSGGTAALGCLVKDYFPEPVTVSWNSGALTSGVHTFPAVLQSSGLYSLSSVVTVPSSSLGTQTYICNVNHKPSNTKVDKKVEPKSCDKTHTCPPCPAPELLGGPSVFLFPPKPKDTLMISRTPEVTCVVVDVSHEDPEVKFNWYVDGVEVHNAKTKPREEQYNSTYRVVSVLTVLHQDWLNGKEYKCKVSNKALPAPIEKTISKAKGQPREPQVYTLPPSRDELTKNQVSLTCLVKGFYPSDIAVEWESNGQPENNYKTTPPVLDSDGSFFLYSKLTVDKSRWQQGNVFSCSVMHEALHNHYTQKSLSLSPGKEIVLTQSPGTLSLSPGERATLSCRASGNIHSYLAWYQQKPGQAPRLLIYNAKTLADGIPDRFSGSGSGTDYTLTISRLEPEDFAVYYCQHFWNTPPTFGAGTKLELKRTVAAPSVFIFPPSDEQLKSGTASVVCLLNNFYPREAKVQWKVDNALQSGNSQESVTEQDSKDSTYSLSSTLTLSKADYEKHKVYACEVTHQGLSSPVTKSFNRGEC

SEQ ID NO: 45 - protein, 663 aa, Artificial Sequence; identical to SEQ ID NO: 41
  Synthetic polypeptide

SEQ ID NO: 46 - protein, 663 aa, Artificial Sequence; identical to SEQ ID NO: 42
  Synthetic polypeptide

SEQ ID NO: 47 - protein, 663 aa, Artificial Sequence; identical to SEQ ID NO: 43
  Synthetic polypeptide

SEQ ID NO: 48 - protein, 663 aa, Artificial Sequence; identical to SEQ ID NO: 44
  Synthetic polypeptide

SEQ ID NO: 49 - protein, 116 aa, Homo sapiens
EVQLVESGGGLVKPGGSLRLSCAASGFTFRSYSMNWVRQAPGKGLEWVSSIISSSSYIYYADSVKGRFTISRDNAKNSLYLQMNSLRAEDTALYYCARDQNAMDVWGQGTTVTVSS

SEQ ID NO: 50 - protein, 215 aa, Homo sapiens
SYELTQPPSVSVAPGKTARITCAGNNIGSKSVHWYQQKPGQAPVLVIYYDSDRPSGIPERFSGSNSGNTATLTISRVEAGDEADYYCQVWDSGSDHPWVFGGGTKLTVLRQPKAAPSVTLFPPSSEELQANKATLVCLISDFYPGAVTVAWKADSSPVKAGVETTTPSKQSNNKYAASSYLSLTPEQWKSHRSYSCQVTHEGSTVEKTVAPTECS

SEQ ID NO: 51 - protein, 569 aa, Homo sapiens
EVQLVESGGGLVKPGGSLRLSCAASGFTFSGYSMNWVRQAPGKGLEWVSSISSSSTYIYYVDSVRGRFTISRDNAKNSLYLQMNSLRAEDTAVYYCARDENDMDVWGQGTTVTVSSGSASAPTLFPLVSCENSPSDTSSVAVGCLAQDFLPDSITFSWKYKNNSDISSTRGFPSVLRGGKYAATSQVLLPSKDVMQGTDEHVVCKVQHPNGNKEKNVPLPVIAELPPKVSVFVPPRDGFFGNPRKSKLICQATGFSPRQIQVSWLREGKQVGSGVTTDQVQAEAKESGPTTYKVTSTLTIKESDWLSQSMFTCRVDHRGLTFQQNASSMCVPDQDTAIRVFAIPPSFASIFLTKSTKLTCLVTDLTTYDSVTISWTRQNGEAVKTHTNISESHPNATFSAVGEASICEDDWNSGERFTCTVTHTDLPSPLKQTISRPKGVALHRPDVYLLPPAREQLNLRESATITCLVTGFSPADVFVQWMQRGQPLSPEKYVTSAPMPEPQAPGRYFAHSILTVSEEEWNTGETYTCVVAHEALPNRVTERTVDKSTGKPTLYNVSLVMSDTAGTCY

SEQ ID NO: 52 - protein, 215 aa, Homo sapiens
SYVLTQPPSVSVAPGKTARITCGGNNIGTKSVHWYQQKPGQAPVLVIYYDSDRPSGIPERFSGSNSGNTATLTISRVEAGDEADYYCQVWDSGSDHPWVFGGGTKLTVLRQPKAAPSVTLFPPSSEELQANKATLVCLISDFYPGAVTVAWKADSSPVKAGVETTTPSKQSNNKYAASSYLSLTPEQWKSHRSYSCQVTHEGSTVEKTVAPTECS

SEQ ID NO: 53 - protein, 110 aa, Homo sapiens
SYELTQPPSVSVAPGKTARITCAGNNIGSKSVHWYQQKPGQAPVLVIYYDSDRPSGIPERFSGSNSGNTATLTISRVEAGDEADYYCQVWDSGSDHPWVFGGGTKLTVLR